European Patent Specification EP 3 107 374 B1, published October 16, 2024. Title: Hybrid BW-Type Mushroom Strains and Lines and Methods and Uses Therefor. Applicant: Sylvan America, Inc. The sequence listing filed with the application follows.

SEQUENCE LISTING (12 sequences)

SEQ ID NO: 1 - DNA, 18 bp, Agaricus bisporus
aggcrycccatcttcasc

SEQ ID NO: 2 - DNA, 17 bp, Agaricus bisporus
gttcgacgacggactgc

SEQ ID NO: 3 - DNA, 19 bp, Agaricus bisporus
tccgtaggtgaacctgcgg

SEQ ID NO: 4 - DNA, 20 bp, Agaricus bisporus
tcctccgcttattgatatgc

SEQ ID NO: 5 - DNA, 23 bp, Agaricus bisporus
aytcrcaamaacataccttcaac

SEQ ID NO: 6 - DNA, 18 bp, Agaricus bisporus
cattcggcgattttctca

SEQ ID NO: 7 - DNA, 21 bp, Agaricus bisporus
gacgatgcgggactggtggat

SEQ ID NO: 8 - DNA, 23 bp, Agaricus bisporus
ggtctggcctacrggagtgttgt

SEQ ID NO: 9 - DNA, 23 bp, Agaricus bisporus
ccgccagcacaaggaatcaaatg

SEQ ID NO: 10 - DNA, 23 bp, Agaricus bisporus
tcagtcggccctcaaaacagtcg

SEQ ID NO: 11 - DNA, 22 bp, Agaricus bisporus
tcgggtggttgcaactgaaaag

SEQ ID NO: 12 - DNA, 24 bp, Agaricus bisporus
ttcctttccgccttaattgtttct